European Patent Specification EP 2 451 268 B1, published May 6, 2026. Title: METHOD TO DEVELOP HIGH OLEIC ACID SOYBEANS USING CONVENTIONAL SOYBEAN BREEDING TECHNIQUES. Applicant: University of Missouri United States Department of Agriculture. Application US 12/832,760. The sequence listing filed with the application follows.

SEQUENCE LISTING (19 sequences)

SEQ ID NO: 1 - DNA, 1104 bp, Glycine max
  CDS (1)..(1104): nucleotide sequence of FAD2-1B mutant PI 283327
  mutation (66)..(66): G to A mutation (silent mutation)
  mutation (257)..(257): C to T mutation resulting in an amino acid substitution of Serine to Phenylalanine at amino acid 86
  mutation (376)..(376): A to G mutation resulting in an amino acid substitution of Methionine to Valine at amino acid 126
  mutation (410)..(410): C to G mutation leading to a corresponding amino acid mutation from Proline to Arginine at amino acid 137
  mutation (657)..(657): C to T mutation (silent mutation)
  mutation (669)..(669): T to C mutation (silent mutation)
  mutation (682)..(682): T to C mutation (silent mutation)
  mutation (918)..(918): A to G mutation (silent mutation)
atgggtctagcaaaggaaacaataatgggaggtggaggccgtgtggccaaagttgaaattcagcaaaagaagcctctctcaagggttccaaacacaaagccaccattcactgttggccaactcaagaaagccattccaccgcactgctttcagcgttccctcctcacttcattgtcctatgttgtttatgacctttcattggctttcattttctacattgccaccacctacttccacctcctccctcacccctttttcctcattgcatggccaatctattgggttctccaaggttgcattcttactggcgtgtgggtgattgctcacgagtgtggtcaccatgccttcagcaagtacccatgggttgatgatgttgtgggtttgaccgttcactcagcacttttagtccgttatttctcatggaaaataagccatcgccgccaccactccaacacgggttcccttgaccgtgatgaagtgtttgtcccaaaaccaaaatccaaagttgcatggtacaccaagtacctgaacaaccctctaggaagggctgcttctcttctcatcacactcacaatagggtggcctttgtatttagccttcaatgtctctggcagaccctatgatggttttgctagccactaccacccttatgctcctatatattcaaaccgtgagaggcttctgatctatgtctctgatgttgctttgttttctgtgacttacttgctctaccgtgttgcaactatgaaagggttggtttggctgctatgtgtttatggggtgccattgctcattgtgaacggttttcttgtgaccatcacatatctgcagcacacacactatgccttgcctcactatgattcatcagaatgggattggctgaggggtgctttggcaactatggacagagattatgggattctgaacaaggtgtttcaccacataactgatactcatgtggctcaccatcttttctctacaatgccatttgatgacacaccattttacaaggcactgtggagagaagcaagagagtgcctctatgtggagccagatgaaggaacatccgagaagggcgtgtattggtacaggaacaagtattga

SEQ ID NO: 2 - protein, 367 aa, Glycine max
  amino acid sequence of FAD2-1B mutant PI 283327
MGLAKETIMGGGGRVAKVEIQQKKPLSRVPNTKPPFTVGQLKKAIPPHCFQRSLLTSLSYVVYDLSLAFIFYIATTYFHLLPHPFFLIAWPIYWVLQGCILTGVWVIAHECGHHAFSKYPWVDDVVGLTVHSALLVRYFSWKISHRRHHSNTGSLDRDEVFVPKPKSKVAWYTKYLNNPLGRAASLLITLTIGWPLYLAFNVSGRPYDGFASHYHPYAPIYSNRERLLIYVSDVALFSVTYLLYRVATMKGLVWLLCVYGVPLLIVNGFLVTITYLQHTHYALPHYDSSEWDWLRGALATMDRDYGILNKVFHHITDTHVAHHLFSTMPFDDTPFYKALWREARECLYVEPDEGTSEKGVYWYRNKY

SEQ ID NO: 3 - DNA, 1164 bp, Glycine max
  CDS (1)..(1164): nucleotide sequence of FAD2-1B mutant PI 567189A
  mutation (66)..(66): G to A mutation (silent mutation)
  mutation (257)..(257): C to T mutation resulting in an amino acid substitution of Serine to Phenylalanine at amino acid 86
  mutation (376)..(376): A to G mutation resulting in an amino acid substitution of Methionine to Valine at amino acid 126
  mutation (428)..(428): T to C mutation resulting in corresponding amino acid substitution of Isoleucine to Threonine at amino acid 143
  mutation (657)..(657): C to T mutation (silent mutation)
  mutation (669)..(669): T to C mutation (silent mutation)
  mutation (682)..(682): T to C mutation (silent mutation)
  mutation (918)..(918): A to G mutation (silent mutation)
atgggtctagcaaaggaaacaataatgggaggtggaggccgtgtggccaaagttgaaattcagcaaaagaagcctctctcaagggttccaaacacaaagccaccattcactgttggccaactcaagaaagccattccaccgcactgctttcagcgttccctcctcacttcattgtcctatgttgtttatgacctttcattggctttcattttctacattgccaccacctacttccacctcctccctcacccctttttcctcattgcatggccaatctattgggttctccaaggttgcattcttactggcgtgtgggtgattgctcacgagtgtggtcaccatgccttcagcaagtacccatgggttgatgatgttgtgggtttgaccgttcactcagcacttttagtcccttatttctcatggaaaacaagccatcgccgccaccactccaacacgggttcccttgaccgtgatgaagtgtttgtcccaaaaccaaaatccaaagttgcatggtacaccaagtacctgaacaaccctctaggaagggctgcttctcttctcatcacactcacaatagggtggcctttgtatttagccttcaatgtctctggcagaccctatgatggttttgctagccactaccacccttatgctcctatatattcaaaccgtgagaggcttctgatctatgtctctgatgttgctttgttttctgtgacttacttgctctaccgtgttgcaactatgaaagggttggtttggctgctatgtgtttatggggtgccattgctcattgtgaacggttttcttgtgaccatcacatatctgcagcacacacactatgccttgcctcactatgattcatcagaatgggattggctgaggggtgctttggcaactatggacagagattatgggattctgaacaaggtgtttcaccacataactgatactcatgtggctcaccatcttttctctacaatgccacattaccatgcaacggaggcaaccaatgcaatgaagccaatattgggtgagtactaccgatttgatgacacaccattttacaaggcactgtggagagaagcaagagagtgcctctatgtggagccagatgaaggaacatccgagaagggcgtgtattggtacaggaacaagtattga

SEQ ID NO: 4 - protein, 387 aa, Glycine max
  amino acid sequence of FAD2-1B mutant PI 567189A
MGLAKETIMGGGGRVAKVEIQQKKPLSRVPNTKPPFTVGQLKKAIPPHCFQRSLLTSLSYVVYDLSLAFIFYIATTYFHLLPHPFFLIAWPIYWVLQGCILTGVWVIAHECGHHAFSKYPWVDDVVGLTVHSALLVPYFSWKTSHRRHHSNTGSLDRDEVFVPKPKSKVAWYTKYLNNPLGRAASLLITLTIGWPLYLAFNVSGRPYDGFASHYHPYAPIYSNRERLLIYVSDVALFSVTYLLYRVATMKGLVWLLCVYGVPLLIVNGFLVTITYLQHTHYALPHYDSSEWDWLRGALATMDRDYGILNKVFHHITDTHVAHHLFSTMPHYHATEATNAMKPILGEYYRFDDTPFYKALWREARECLYVEPDEGTSEKGVYWYRNKY

SEQ ID NO: 5 - DNA, 1357 bp, Glycine max
  CDS (74)..(1237)
tatttgcattgtattgatagcccctccattcccaagagtataaaactgcatcgaataatacaagccactaggcatgggtctagcaaaggaaacaacaatgggaggtagaggtcgtgtggccaaagtggaagttcaagggaagaagcctctctcaagggttccaaacacaaagccaccattcactgttggccaactcaagaaagcaattccaccacactgctttcagcgctccctcctcacttcattctcctatgttgtttatgacctttcatttgccttcattttctacattgccaccacctacttccacctccttcctcaacccttttccctcattgcatggccaatctattgggttctccaaggttgccttctcactggtgtgtgggtgattgctcacgagtgtggtcaccatgccttcagcaagtaccaatgggttgatgatgttgtgggtttgacccttcactcaacacttttagtcccttatttctcatggaaaataagccatcgccgccatcactccaacacaggttcccttgaccgtgatgaagtgtttgtcccaaaaccaaaatccaaagttgcatggttttccaagtacttaaacaaccctctaggaagggctgtttctcttctcgtcacactcacaatagggtggcctatgtatttagccttcaatgtctctggtagaccctatgatagttttgcaagccactaccacccttatgctcccatatattctaaccgtgagaggcttctgatctatgtctctgatgttgctttgttttctgtgacttactctctctaccgtgttgcaaccctgaaagggttggtttggctgctatgtgtttatggggtgcctttgctcattgtgaacggttttcttgtgactatcacatatttgcagcacacacactttgccttgcctcattacgattcatcagaatgggactggctgaagggagctttggcaactatggacagagattatgggattctgaacaaggtgtttcatcacataactgatactcatgtggctcaccatctcttctctacaatgccacattaccatgcaatggaggcaaccaatgcaatcaagccaatattgggtgagtactaccaatttgatgacacaccattttacaaggcactgtggagagaagcgagagagtgcctctatgtggagccagatgaaggaacatccgagaagggcgtgtattggtacaggaacaagtattgatggagcaaccaatgggccatagtgggagttatggaagttttgtcatgtattagtacataattagtagaatgttataaataagtggatttgccgcgtaatgactttgtgtgtattgtgaaa

SEQ ID NO: 6 - protein, 387 aa, Glycine max
MGLAKETTMGGRGRVAKVEVQGKKPLSRVPNTKPPFTVGQLKKAIPPHCFQRSLLTSFSYVVYDLSFAFIFYIATTYFHLLPQPFSLIAWPIYWVLQGCLLTGVWVIAHECGHHAFSKYQWVDDVVGLTLHSTLLVPYFSWKISHRRHHSNTGSLDRDEVFVPKPKSKVAWFSKYLNNPLGRAVSLLVTLTIGWPMYLAFNVSGRPYDSFASHYHPYAPIYSNRERLLIYVSDVALFSVTYSLYRVATLKGLVWLLCVYGVPLLIVNGFLVTITYLQHTHFALPHYDSSEWDWLKGALATMDRDYGILNKVFHHITDTHVAHHLFSTMPHYHAMEATNAIKPILGEYYQFDDTPFYKALWREARECLYVEPDEGTSEKGVYWYRNKY

SEQ ID NO: 7 - DNA, 1164 bp, Glycine max
  CDS (1)..(1104)
  mutation (350)..(350): X to A mutation resulting in a corresponding amino acid subsituttion of Serine to Asparagine at amino acid position 117
atgggtctagcaaaggaaacaacaatgggaggtagaggtcgtgtggccaaagtggaagttcaagggaagaagcctctctcaagggttccaaacacaaagccaccattcactgttggccaactcaagaaagcaattccaccacactgctttcagcgctccctcctcacttcattctcctatgttgtttatgacctttcatttgccttcattttctacattgccaccacctacttccacctccttcctcaacccttttccctcattgcatggccaatctattgggttctccaaggttgccttctcactggtgtgtgggtgattgctcacgagtgtggtcaccatgccttcaacaagtaccaatgggttgatgatgttgtgggtttgacccttcactcaacacttttagtcccttatttctcatggaaaataagccatcgccgccatcactccaacacaggttcccttgaccgtgatgaagtgtttgtcccaaaaccaaaatccaaagttgcatggttttccaagtacttaaacaaccctctaggaagggctgtttctcttctcgtcacactcacaatagggtggcctatgtatttagccttcaatgtctctggtagaccctatgatagttttgcaagccactaccacccttatgctcccatatattctaaccgtgagaggcttctgatctatgtctctgatgttgctttgttttctgtgacttactctctctaccgtgttgcaaccctgaaagggttggtttggctgctatgtgtttatggggtgcctttgctcattgtgaacggttttcttgtgactatcacatatttgcagcacacacactttgccttgcctcattacgattcatcagaatgggactggctgaagggagctttggcaactatggacagagattatgggattctgaacaaggtgtttcatcacataactgatactcatgtggctcaccatctcttctctacaatgccacattaccatgcaatggaggcaaccaatgcaatcaagccaatattgggtgagtactaccaatttgatgacacaccattttacaaggcactgtggagagaagcgagagagtgcctctatgtggagccagatgaaggaacatccgagaagggcgtgtattggtacaggaacaagtattga

SEQ ID NO: 8 - protein, 368 aa, Glycine max
MGLAKETTMGGRGRVAKVEVQGKKPLSRVPNTKPPFTVGQLKKAIPPHCFQRSLLTSFSYVVYDLSFAFIFYIATTYFHLLPQPFSLIAWPIYWVLQGCLLTGVWVIAHECGHHAFNKYQWVDDVVGLTLHSTLLVPYFSWKISHRRHHSNTGSLDRDEVFVPKPKSKVAWFSKYLNNPLGRAVSLLVTLTIGWPMYLAFNVSGRPYDSFASHYHPYAPIYSNRERLLIYVSDVALFSVTYSLYRVATLKGLVWLLCVYGVPLLIVNGFLVTITYLQHTHFALPHYDSSEWDWLKGALATMDRDYGILNKVFHHITDTHVAHHLFSTMPHYHAMEATNAIKPILGEYYQFDDTPFYKALWREARECLY

SEQ ID NO: 9 - DNA, 1164 bp, Glycine max
  CDS (1)..(1104)
atgggtctagcaaaggaaacaacaatgggaggtagaggtcgtgtggccaaagtggaagttcaagggaagaagcctctctcaagggttccaaacacaaagccaccattcactgttggccaactcaagaaagcaattccaccacactgctttcagcgctccctcctcacttcattctcctatgttgtttatgacctttcatttgccttcattttctacattgccaccacctacttccacctccttcctcaacccttttccctcattgcatggccaatctattgggttctccaaggttgccttctcactggtgtgtgggtgattgctcacgagtgtggtcaccatgccttcagcaagtaccaatgggttgatgatgttgtgggtttgacccttcactcaacacttttagtcccttatttctcatggaaaataagccatcgccgccatcactccaacacaggttcccttgaccgtgatgaagtgtttgtcccaaaaccaaaatccaaagttgcatggttttccaagtacttaaacaaccctctaggaagggctgtttctcttctcgtcacactcacaatagggtggcctatgtatttagccttcaatgtctctggtagaccctatgatagttttgcaagccactaccacccttatgctcccatatattctaaccgtgagaggcttctgatctatgtctctgatgttgctttgttttctgtgacttactctctctaccgtgttgcaaccctgaaagggttggtttggctgctatgtgtttatggggtgcctttgctcattgtgaacggttttcttgtgactatcacatatttgcagcacacacactttgccttgcctcattacgattcatcagaatgggactggctgaagggagctttggcaactatggacagagattatgggattctgaacaaggtgtttcatcacataactgatactcatgtggctcaccatctcttctctacaatgccacattaccatgcaatggaggcaaccaatgcaatcaagccaatattgggtgagtactaccaatttgatgacacaccattttacaaggcactgtggagagaagcgagagagtgcctctatgtggagccagatgaaggaacatccgagaagggcgtgtattggtacaggaacaagtattga

SEQ ID NO: 10 - protein, 368 aa, Glycine max
MGLAKETTMGGRGRVAKVEVQGKKPLSRVPNTKPPFTVGQLKKAIPPHCFQRSLLTSFSYVVYDLSFAFIFYIATTYFHLLPQPFSLIAWPIYWVLQGCLLTGVWVIAHECGHHAFSKYQWVDDVVGLTLHSTLLVPYFSWKISHRRHHSNTGSLDRDEVFVPKPKSKVAWFSKYLNNPLGRAVSLLVTLTIGWPMYLAFNVSGRPYDSFASHYHPYAPIYSNRERLLIYVSDVALFSVTYSLYRVATLKGLVWLLCVYGVPLLIVNGFLVTITYLQHTHFALPHYDSSEWDWLKGALATMDRDYGILNKVFHHITDTHVAHHLFSTMPHYHAMEATNAIKPILGEYYQFDDTPFYKALWREARECLY

SEQ ID NO: 11 - DNA, 1164 bp, Glycine max
  CDS (1)..(1104)
atgggtctagcaaaggaaacaataatgggaggtggaggccgtgtggccaaagttgaaattcagcagaagaagcctctctcaagggttccaaacacaaagccaccattcactgttggccaactcaagaaagccattccaccgcactgctttcagcgttccctcctcacttcattgtcctatgttgtttatgacctttcattggctttcattttctacattgccaccacctacttccacctcctccctcaccccttttccctcattgcatggccaatctattgggttctccaaggttgcattcttactggcgtgtgggtgattgctcacgagtgtggtcaccatgccttcagcaagtacccatgggttgatgatgttatgggtttgaccgttcactcagcacttttagtcccttatttctcatggaaaataagccatcgccgccaccactccaacacgggttcccttgaccgtgatgaagtgtttgtcccaaaaccaaaatccaaagttgcatggtacaccaagtacctgaacaaccctctaggaagggctgcttctcttctcatcacactcacaatagggtggcctttgtatttagccttcaatgtctctggcagaccctatgatggttttgctagccactaccacccttatgctcccatatattcaaatcgtgagaggcttttgatctatgtctctgatgttgctttgttttctgtgacttacttgctctaccgtgttgcaactatgaaagggttggtttggctgctatgtgtttatggggtgccattgctcattgtgaacggttttcttgtgaccatcacatatctgcagcacacacactatgccttgcctcactatgattcatcagaatgggattggctgaggggtgctttggcaactatggacagagattatggaattctgaacaaggtgtttcaccacataactgatactcatgtggctcaccatcttttctctacaatgccacattaccatgcaacggaggcaaccaatgcaatgaagccaatattgggtgagtactaccgatttgatgacacaccattttacaaggcactgtggagagaagcaagagagtgcctctatgtggagccagatgaaggaacatccgagaagggcgtgtattggtacaggaacaagtattga

SEQ ID NO: 12 - protein, 368 aa, Glycine max
MGLAKETIMGGGGRVAKVEIQQKKPLSRVPNTKPPFTVGQLKKAIPPHCFQRSLLTSLSYVVYDLSLAFIFYIATTYFHLLPHPFSLIAWPIYWVLQGCILTGVWVIAHECGHHAFSKYPWVDDVMGLTVHSALLVPYFSWKISHRRHHSNTGSLDRDEVFVPKPKSKVAWYTKYLNNPLGRAASLLITLTIGWPLYLAFNVSGRPYDGFASHYHPYAPIYSNRERLLIYVSDVALFSVTYLLYRVATMKGLVWLLCVYGVPLLIVNGFLVTITYLQHTHYALPHYDSSEWDWLRGALATMDRDYGILNKVFHHITDTHVAHHLFSTMPHYHATEATNAMKPILGEYYRFDDTPFYKALWREARECLY

SEQ ID NO: 13 - DNA, 22 bp, Artificial
  forward primer for FAD2-1A
actgcatcgaataatacaagcc

SEQ ID NO: 14 - DNA, 19 bp, Artificial
  reverse primer for FAD2-1A
tgatattgtcccgtgcagc

SEQ ID NO: 15 - DNA, 20 bp, Artificial
  forward primer for FAD2-1B
cccgctgtcccttttaaact

SEQ ID NO: 16 - DNA, 25 bp, Artificial
  reverse primer for FAD2-1B
ttacattatagccatggatcgctac

SEQ ID NO: 17 - DNA, 28 bp, Artificial
  SimpleProbe GmFAD2-1B
agtcccttatttctcatggaaaataagc

SEQ ID NO: 18 - DNA, 22 bp, Artificial
  primer for genotyping reactions
actgcatcgaataatacaagcc

SEQ ID NO: 19 - DNA, 19 bp, Artificial
  primer for genotyping reactions
tgatattgtcccgtccagc